European Patent Application EP 4 656 721 A1, published December 3, 2025. Title: HSP60 PROTEINS OBTAINED BY MEANS OF ANCESTRAL SEQUENCE RECONSTRUCTION (ASR). Applicant: INSTITUTO NACIONAL DE TECNICA AEROESPACIAL. The sequence listing filed with the application follows.

SEQUENCE LISTING (12 sequences)

SEQ ID NO: 1 - protein, 532 aa, synthetic construct
MTSSGIKFGEEARRALVRGVNQLADLVKATLGPKGRNVVLEEKFGHVTITNDGATVARRISLPDPFENMGAKLVREVARRTNEEVGDGTTTAVVLAGALVREGHKLIAAGLNPMRLVKGMRKAVELVCEELKRLALPVDGLEELAGVARTAAKDEEIAELIAEAMEKLGPDGIIEVEESKGAETHLELVEGVHFDKGLLSPYFVTEAEKMSAELEDPRIAITDKPISDAEELLPVLEACVQTGRKLLIVANDISGEALAMLVANKLRGKVNVVAVKAPGTGEQRKDALEDLAALTGGRVISEVAGLTLEDVTPDDLGRARRVRVTRDNFTIIGGAGDKEEIEERVKQLKARLAATSDDEDREKLQERLARLSGGIAVIKVGAATETELEERKHRVEDAVNAVQAAVESGVVPGGGAALLRCARALEDLAEAENDEEKAGVRAVAKALEEPLRQIVENAGRDPAEVLDKVKEADPDLGYDVLTGEFVDMWEAGIIDPAPVTRSALQTAVSVASMLLTTEALVHKKRPEEAAAP

SEQ ID NO: 2 - protein, 540 aa, synthetic construct
MAKQIKFDTDARNALLRGVDKLADAVKVTLGPKGRNVIIEKKFGAPTITKDGVTVAKEIELEDPFENMGAQMVKEVASKTSDVAGDGTTTATVLAQAIVREGLKNVAAGANPMDLKRGIDKAVEAVVEELKKMAKPVNGKEEIAQVATISANNDPEIGKLIAEAMEKVGKDGVITVEESKSTETTLDVVEGMQFDRGYLSPYFVTDSEKMEAVLENPYILIYDKKISNMKDLLPILEKVAQSGKPLLIIAEDVEGEALATLVVNKLRGTLKVCAVKAPGFGDRRKAMLEDIAILTGGTVISEETGYKLENATLDYLGRAKRVTIDKDNTTIVDGAGDKEDIKARVNQIKKQIENTTSDYDREKLQERLAKLAGGVAVIKVGAATEVEMKEKKARVEDALHATRAAVEEGIVPGGGVALIRAAKALENLEGENGDQKTGVKIVRRALEEPLRQIVANAGLEGSVVVNKVKEGKGNFGYNARTEEYDLIEAGVIDPAKVTRTALQNAASIAGMLLTTECVITEKPELEEAPPMPGGGMGGMM

SEQ ID NO: 3 - protein, 530 aa, synthetic construct
MGQPMVVLSENTERTSGRDARKNNIAAARAIADMVKTTLGPRGMNKMLVNSLGDVTITNDGATILEEMDIEHPAAKMLKEVAKAQEEEAGDGTTTAVVLAGALLEEAEKLIEQGIHPTTIIKGYRKAVDKALEVLEEVAIPVDPDDEETLKAVARTAMTGKASEENREEIADLVVEAVLSLAEDGGGKYRVDLDNIKIEKQTGGGASDTELIEGVVLDKEPVHEDMPKKLENAKVAVLDAPIEVEKTELDAKISISSPEQFQAFLDQEEKQLREMVDKIVDTGANVVFCEKGIDDQVEHMLAKKGILAVRRVKKDDLEKIAKATGARVVSNIDELTPEDLGHAGLVEQRKKGEDRMVFVSGCKNEPVATILIRAATEHVVEELERAIDDALNAVKAAIKDGKVVPGGGAAEVAVARKLREYAKSLSGKEQLAIEAFADALEEIPRTLAENAGLDPIDTLVQLRAAHEEGDKNIGIDCLTGEVADMLEAGVIDPAAVKKQAIKSATEAATMILRIDDIIPAKAPTGEDGDG

SEQ ID NO: 4 - protein, 518 aa, synthetic construct
MPLKQASSNTEADERFQALLTNVNAVRAIADAVEGTLGPKGLDVMLVDKFGEVTITNDGVTILDQMDVQHPAARMLIQVARAQEEEVGDGTTTATVLAGALVSEGVNQVEQGVPVSRVIEGLRRGVERALELLRKQALPVEGLDDPRLRAVARIAAREREDIADLVVEAARHIGEDKLQDPNFKLADTVTAREGAENQVIEGVVLNKQPLNKEMPKKLEDARVLVLDDPLEPEEIDEEALSTEAGFARYLEAQEEFRENLEKLVELGVKLVLCEKGIDDTAEELLAEAGIMAIQRVSRKDLERVAEFTGARPVKRTALNKDAEELAKLLGHAERVRYDEKLEHVCLSGGSGEPIATVLVGAATEEVVGERERVAKDAASAVQAAIRGGVVPGGGAAELAVAREVEKLAEEVKGMERYGVEAVAEALKKPLRQIVANAGFNPLEKLGDLRAAHRTGNDSLGIDCDTGEVVDMWEAGVIDPAPVKLHALKAAGEVAAAILRINTIIKMKETGPDGGEDRG

SEQ ID NO: 5 - protein, 548 aa, Escherichia coli
MAAKDVKFGNDARVKMLRGVNVLADAVKVTLGPKGRNVVLDKSFGAPTITKDGVSVAREIELEDKFENMGAQMVKEVASKANDAAGDGTTTATVLAQAIITEGLKAVAAGMNPMDLKRGIDKAVTAAVEELKALSVPCSDSKAIAQVGTISANSDETVGKLIAEAMDKVGKEGVITVEDGTGLQDELDVVEGMQFDRGYLSPYFINKPETGAVELESPFILLADKKISNIREMLPVLEAVAKAGKPLLIIAEDVEGEALATLVVNTMRGIVKVAAVKAPGFGDRRKAMLQDIATLTGGTVISEEIGMELEKATLEDLGQAKRVVINKDTTTIIDGVGEEAAIQGRVAQIRQQIEEATSDYDREKLQERVAKLAGGVAVIKVGAATEVEMKEKKARVEDALHATRAAVEEGVVAGGGVALIRVASKLADLRGQNEDQNVGIKVALRAMEAPLRQIVLNCGEEPSVVANTVKGGDGNYGYNAATEEYGNMIDMGILDPTKVTRSALQYAASVAGLMITTECMVTDLPKNDAADLGAAGGMGGMGGMGGMM

SEQ ID NO: 6 - protein, 545 aa, Chlorobaculum tepidum
MTAKDILFDAEARTKLKVGVDKLANAVKVTLGPAGRNVLIDKKFGAPTSTKDGVTVAKEIELVDPVENMGAQMVREVASKTSDVAGDGTTTATVLAQAIYREGLKNVTAGARPIDLKRGIDRAVKEVVAELRNISRSISGKKEIAQVGTISANNDPEIGELIAEAMDKVGKDGVITVEEAKGMETELKVVEGMQFDRGYLSPYFVTNSETMEAELDEALILIHDKKISNMKELLPILEKAAQSGRPLLIIAEDIEGEALATLVVNKLRGTLKVAAVKAPGFGDRRKAMLEDIAILTGGTVISEEKGYKLENATMAYLGQAARITIDKDNTTIVEGKGKQEEIKARINEIKGQIEKSTSDYDTEKLQERLAKLSGGVAVLKIGASTEVEMKEKKARVEDALHATRAAVQEGIVVGGGVALIRAAKGLAKAVADNEDQKTGIEIIRRALEEPLRQIVANTGTTDGAVVLEKVKNAEGDYGFNARTEQYENLIEAGVVDPTKVTRSALENAASVASILLTTEAAITDVKEDKADMPAMPPGGMGGGMY

SEQ ID NO: 7 - protein, 548 aa, Thermococcus sp.
MAQLSGQPVVILPEGTQRYVGRDAQRLNILAARIIAETVRTTLGPKGMDKMLVDSLGDIVVTNDGATILDKIDLQHPAAKMMVEVAKTQDKEAGDGTTTAVVIAGELLRKAEELLDQNIHPSIIIKGYALAAEKAQEILDEIAIRVDPDDEETLLKIAATSITGKNAESHKELLAKLAVEAVKQVAEKKDGKYVVDLDNIKFEKKAGEGVEESELVRGVVIDKEVVHPRMPKRVENAKIALINEALEVKKTETDAKINITSPDQLMSFLEQEEKMLKDMVDHIAQTGANVVFVQKGIDDLAQHYLAKYGIMAVRRVKKSDMEKLAKATGAKIVTNVKDLTPEDLGYAEVVEERKLAGENMIFVEGCKNPKAVTILIRGGTEHVIDEVERALEDAVKVVKDVMEDGAVLPAGGAPEIELAIRLDEYAKQVGGKEALAIENFADALKIIPKTLAENAGLDTVEMLVKVISEHKNRGLGIGIDVFEGKPADMLEKGIIEPLRVKKQAIKSASEAAIMILRIDDVIAAKATKPEGGQGGGMPGGMGGMDMGM

SEQ ID NO: 8 - protein, 521 aa, Carboxydothermus hydrogenoformans
MKKENQTQEIEERYQALFSNAAAVKALTQVVANSLGPKGLDAMLVDRFGEVVVTNDGVTILTLMDAQHPAARMVVNMARAQEREVGDGTTTAAVLAGALVSEGVNQILKGVPVSKVLAGMNRALNHALFLIRKNAIKVGSITDDRLLAAAKIAGRGDERVAAILRDAAAMLEDKLQDPGFKLADLVLAKVGADTTLIPGVVINKSPLWEEGSQKLQEVRLLVLDDGLYPEEVEEEALASEAGFEQYLKNQKIFQENLKKLKELGVKLILLTRGISDIAEEFCYENEIMVITRITQKELKRVLEFTGARAAKRTSLNKPVEELQKMLGYARTCFYDSRLDFTIIEGGAGKATATVLIGAATDEVVDEQERIAKDAAGSFAAAYRSGVLPGGGAFFLYLSREVESLKNRLPGMESYGVMAFSEALKVPFRVMAENAGFNGLEKLGDLMTLQVQKNNYALGLDFETGEFIDMIAGGVVDPAEVVYQAVKNASEVAISLLKINTIIKMKDYEVLKEGEQEDGGKR

SEQ ID NO: 9 - DNA, 1599 bp, synthetic construct
  source 1..1599: mol_type = other DNA
atgaccagcagcggcatcaagtttggcgaggaagcgcgtcgtgcgctggtgcgtggcgttaaccagctggcggatctggtgaaggcgaccctgggtccgaaaggtcgtaacgtggttctggaggaaaagttcggccacgtgaccatcaccaacgatggtgcgaccgttgcgcgtcgtattagcctgccggacccgtttgagaacatgggtgcgaaactggtgcgtgaagttgcgcgtcgtaccaacgaggaagtgggcgacggtaccaccaccgcggttgttctggcgggtgcgctggttcgtgagggtcacaaactgattgcggcgggcctgaacccgatgcgtctggttaagggtatgcgtaaagcggtggaactggtttgcgaggaactgaaacgtctggcgctgccggtggatggtctggaagaactggcgggtgttgcgcgtaccgcggcgaaagacgaggaaatcgcggagctgattgcggaggcgatggaaaagctgggcccggacggtatcattgaggtggaggaaagcaagggtgcggaaacccacctggagctggttgagggtgtgcacttcgataagggtctgctgagcccgtactttgttaccgaggcggaaaaaatgagcgcggagctggaagacccgcgtatcgcgattaccgacaagccgatcagcgatgcggaggaactgctgccggtgctggaggcgtgcgttcagaccggccgtaaactgctgatcgtggcgaacgatattagcggtgaagcgctggcgatgctggttgcgaacaagctgcgtggcaaagtgaacgtggttgcggttaaggcgccgggtaccggcgagcaacgtaaagatgcgctggaagatctggcggcgctgaccggtggccgtgtgatcagcgaggttgcgggtctgaccctggaagatgttaccccggatgatctgggtcgtgcgcgtcgtgtgcgtgttacccgtgataacttcaccatcattggtggcgcgggtgacaaagaggagattgaggaacgtgttaagcagctgaaagcgcgtctggcggcgaccagcgatgatgaggatcgtgaaaaactgcaagaacgtctggcgcgtctgagcggtggcattgcggtgattaaggttggcgcggcgaccgagaccgaactggaggaacgtaaacaccgtgttgaggatgcggtgaacgcggttcaggcggcggttgaaagcggtgtggttccgggtggcggtgcggcgctgctgcgttgcgcgcgtgcgctggaggacctggcggaggcggaaaacgatgaggaaaaagcgggcgtgcgtgcggttgcgaaagcgctggaggaaccgctgcgtcaaatcgtggaaaacgcgggtcgtgacccggcggaagtgctggataaggttaaagaagcggacccggatctgggctatgacgtgctgaccggcgagtttgttgatatgtgggaagcgggtatcattgatccggcgccggtgacccgtagcgcgctgcaaaccgctgtgagcgttgcgagcatgctgctgaccaccgaagcgctggttcacaagaaacgtccggaggaagcggcggcgccgtaa

SEQ ID NO: 10 - DNA, 1623 bp, synthetic construct
  source 1..1623: mol_type = other DNA
atggcgaagcaaatcaaattcgacaccgatgcgcgtaacgcgctgctgcgtggtgtggacaagctggcggatgcggttaaagtgaccctgggtccgaagggccgtaacgttatcattgagaagaaattcggtgcgccgaccatcaccaaagacggcgttaccgtggcgaaggagattgaactggaggatccgtttgaaaacatgggtgcgcagatggttaaagaggtggcgagcaaaaccagcgatgtggcgggtgatggtaccaccaccgcgaccgtgctggcgcaagcgatcgttcgtgaaggtctgaaaaacgtggcggcgggtgcgaacccgatggacctgaagcgtggcattgataaagcggttgaggcggtggttgaggaactgaagaaaatggcgaagccggtgaacggtaaagaggaaatcgcgcaggttgcgaccattagcgcgaacaacgacccggaaatcggcaaactgattgcggaagcgatggagaaggttggtaaagatggcgttatcaccgtggaggaaagcaagagcaccgaaaccaccctggacgtggttgagggtatgcaattcgatcgtggctacctgagcccgtattttgtgaccgacagcgaaaaaatggaggcggttctggagaacccgtacatcctgatttatgacaagaaaatcagcaacatgaaggatctgctgccgattctggaaaaagtggcgcagagcggcaagccgctgctgatcattgcggaggatgttgaaggtgaggcgctggcgaccctggtggttaacaaactgcgtggtaccctgaaggtttgcgcggtgaaagcgccgggttttggtgaccgtcgtaaggcgatgctggaagatatcgcgattctgaccggtggcaccgtgatcagcgaggaaaccggttacaagctggagaacgcgaccctggactatctgggccgtgcgaaacgtgtgaccatcgacaaggataacaccaccattgttgatggtgcgggcgacaaggaagatatcaaagcgcgtgttaaccagatcaagaaacaaattgagaacaccaccagcgactacgatcgtgaaaaactgcaagaacgtctggcgaagctggcgggtggcgttgcggtgattaaagtgggtgcggcgaccgaagttgagatgaaggaaaagaaagcgcgtgttgaggatgcgctgcatgcgacccgtgcggcggttgaggaaggcattgtgccgggtggcggtgttgcgctgattcgtgcggcgaaagcgctggaaaacctggaaggcgagaacggcgatcagaagaccggtgttaaaattgtgcgtcgtgcgctggaggaaccgctgcgtcaaattgtggcgaacgcgggtctggaaggcagcgtggttgtgaacaaggttaaagagggtaaaggcaactttggttacaacgcgcgtaccgaggaatatgaagacctgatcgaggcgggcgtgattgatccggcgaaggttacccgtaccgcgctgcagaacgcggcgagcattgcgggtatgctgctgaccaccgagtgcgttattaccgaaaagccggaactggaggaagcgccgccgatgccgggcggtggcatgggtggcatgatg

SEQ ID NO: 11 - DNA, 1590 bp, synthetic construct
  source 1..1590: mol_type = other DNA
atgggccagccgatggtggttctgagcgaaaacaccgagcgtaccagcggtcgtgatgcgcgtaaaaacaacatcgcggcggcgcgtgcgattgcggatatggttaaaaccaccctgggcccgcgtggtatgaacaagatgctggttaacagcctgggcgacgtgaccatcaccaacgatggtgcgaccatcctggaggaaatggacattgaacacccggcggcgaagatgctgaaagaggtggcgaaagcgcaggaagaggaagcgggcgatggtaccaccaccgcggtggttctggcgggtgcgctgctggaagaggcggaaaagctgatcgagcaaggcattcacccgaccaccatcattaagggttaccgtaaagcggttgacaaggcgctggaagtgctggaagaggttgcgatcccggtggatccggacgatgaagagaccctgaaagcggttgcgcgtaccgcgatgaccggcaaggcgagcgaagagaaccgtgaagagattgcggacctggtggttgaagcggttctgagcctggcggaggatggtggcggtaaatatcgtgtggacctggataacatcaagattgaaaaacaaaccggcggtggcgcgagcgacaccgaactgatcgagggtgtggttctggacaaagaaccggttcacgaggatatgccgaagaaactggagaacgcgaaggtggcggttctggacgcgccgattgaagtggagaaaaccgaactggatgcgaagatcagcattagcagcccggagcagttccaagcgtttctggaccaggaagagaaacaactgcgtgaaatggttgacaagatcgtggataccggcgcgaacgtggttttctgcgaaaaaggtatcgacgatcaggttgagcacatgctggcgaagaaaggcattctggcggtgcgtcgtgttaagaaagacgatctggagaagatcgcgaaagcgaccggtgcgcgtgtggttagcaacattgacgaactgaccccggaggatctgggtcatgcgggtctggttgaacagcgtaagaaaggcgaggaccgtatggtgtttgttagcggttgcaagaacgaaccggtggcgaccatcctgattcgtgcggcgaccgaacacgtggttgaagagctggagcgtgcgatcgacgatgcgctgaacgcggtgaaagcggcgattaaggatggtaaagttgttccgggtggcggtgcggcggaagtggcggttgcgcgtaagctgcgtgagtacgcgaaaagcctgagcggcaaggaacagctggcgatcgaggcgttcgcggatgcgctggaagagattccgcgtaccctggcggagaacgcgggtctggacccgatcgataccctggttcaactgcgtgcggcgcacgaagagggcgacaaaaacatcggtattgattgcctgaccggcgaagtggcggacatgctggaggcgggtgttatcgatccggcggcggtgaagaaacaggcgattaaaagcgcgaccgaagcggcgaccatgatcctgcgtattgacgatatcattccggcgaaggcgccgaccggcgaggatggtgatggt

SEQ ID NO: 12 - DNA, 1554 bp, synthetic construct
  source 1..1554: mol_type = other DNA
atgccgctgaagcaggcgagcagcaacaccgaagcggacgagcgtttccaagcgctgctgaccaacgtgaacgcggttcgtgcgattgcggatgcggtggaaggtaccctgggtccgaagggtctggatgtgatgctggttgataaatttggtgaggtgaccatcaccaacgacggcgttaccattctggaccagatggatgttcaacatccggcggcgcgtatgctgatccaggtggcgcgtgcgcaagaggaagaggttggcgatggtaccaccaccgcgaccgtgctggcgggtgcgctggttagcgaaggcgtgaaccaggttgagcaaggtgtgccggttagccgtgtgattgaaggtctgcgtcgtggcgttgaacgtgcgctggagctgctgcgtaaacaggcgctgccggttgagggtctggatgatccgcgtctgcgtgcggttgcgcgtattgcggcgcgtgaacgtgaggacattgcggatctggtggttgaagcggcgcgtcacatcggcgaggacaagctgcaagatccgaacttcaaactggcggacaccgtgaccgcgcgtgagggtgcggagaaccaggttattgaaggcgtggttctgaacaagcaaccgctgaacaaagaaatgccgaagaaactggaggacgcgcgtgtgctggttctggacgatccgctggagccggaagagatcgatgaagaggcgctgagcaccgaagcgggttttgcgcgttacctggaggcgcaggaagagtttcgtgaaaacctggagaaactggtggagctgggtgtgaagctggttctgtgcgagaaaggcattgacgataccgcggaagagctgctggcggaggcgggtatcatggcgattcaacgtgtgagccgtaaagacctggaacgtgttgcggagtttaccggtgcgcgtccggttaagcgtaccgcgctgaacaaagacgcggaagagctggcgaagctgctgggtcacgcggaacgtgtgcgttacgatgaaaaactggagcatgtttgcctgagcggtggcagcggtgaaccgattgcgaccgtgctggttggtgcggcgaccgaagaggtggttggcgaacgtgaacgtgttgcgaaggatgcggcgagcgcggttcaagcggcgattcgtggtggcgtggttccgggtggcggtgcggcggaactggcggtggcgcgtgaagttgagaagctggcggaagaggtgaagggtatggagcgttatggcgtggaagcggttgcggaggcgctgaagaaaccgctgcgtcagatcgttgcgaacgcgggtttcaacccgctggaaaaactgggtgacctgcgtgcggcgcaccgtaccggtaacgatagcctgggcatcgactgcgataccggtgaagtggttgacatgtgggaggcgggcgtgattgatccggcgccggttaagctgcacgcgctgaaagcggcgggtgaggtggcggcggcgatcctgcgtatcaacaccatcatcaagatgaaggaaaccggtccggacggcggtgaggatcgtggc